European Patent Application EP 4 667 573 A1, published December 24, 2025. Title: USE OF MULTIPLE PROMOTERS EFFICIENTLY TARGETED ON ON-BIPOLAR CELLS IN GENE THERAPY TECHNOLOGY. Applicant: Zhongmou Therapeutics Co., Ltd. Application CN. The sequence listing filed with the application follows.

SEQUENCE LISTING (47 sequences)

SEQ ID NO: 1 - DNA, 1061 bp, synthetic construct
  source 1..1061: mol_type = other DNA
tgtgttggttgtaagccagaccccaagaggtggaggtcatgcctccaccctccaaacttccacagccgacaggcctcccagaggaggtggtgggtcctggcctcacagctatgagggctccacagccttctattattttattttcagcttgctggtccttagataaaaatctatctaagacgatgggaatacatggcctgttctctctgagctccagtctgttcccttgcatgtgggaggtgacatgcatgtgcctgtaagagacagaggagggtcggcagcaagggtggtacacttcaggccaggcttgtgctgcaaagacccatgaccccatctgcctttaagaggggcaagacaggcacccctgaaatcagaaatgacacagagagccccacacacagagcagcacagaacagacgggccaccggccacaggatcttcagaagaaggcttgctgtgtcgctgccagattaacggggcgaaaatgcgcactggcagctccaaggagagagctgagacccacagcctgggcctggatgcaaattcttctctgagactcaggcggttggccaggtgggcaccgggcctctgggatctggatgccaccctccaaggggcctcagatgccagcagcaaggggctgtctgccctcgcaatgcgcctttccagacgcccaaatccttcccatttgaccaccctttgcagccaccactttctcaaagtagatttactttcaatctccatttgctaaatctcttccctctaaaccttttggggatggagggattaagcctgattacagatgttgggggtggtagcaggagtcgggcaggaggggccaccaaaagccagcacatgctcctcctaggctgaaccagcctccggccggcctcgccccaggatctcggccccctcgcccagtgcgtggggctgccgccgagtgtggggctgccgccgagtgtgtggctccgctcctgcccacccagggagggcagcccctgtgccactggcctggccacccgagggagtcagcagggtggctcacaggctcactgagagag

SEQ ID NO: 2 - DNA, 750 bp, synthetic construct
  source 1..750: mol_type = other DNA
gctgcaaagacccatgaccccatctgcctttaagaggggcaagacaggcacccctgaaatcagaaatgacacagagagccccacacacagagcagcacagaacagacgggccaccggccacaggatcttcagaagaaggcttgctgtgtcgctgccagattaacggggcgaaaatgcgcactggcagctccaaggagagagctgagacccacagcctgggcctggatgcaaattcttctctgagactcaggcggttggccaggtgggcaccgggcctctgggatctggatgccaccctccaaggggcctcagatgccagcagcaaggggctgtctgccctcgcaatgcgcctttccagacgcccaaatccttcccatttgaccaccctttgcagccaccactttctcaaagtagatttactttcaatctccatttgctaaatctcttccctctaaaccttttggggatggagggattaagcctgattacagatgttgggggtggtagcaggagtcgggcaggaggggccaccaaaagccagcacatgctcctcctaggctgaaccagcctccggccggcctcgccccaggatctcggccccctcgcccagtgcgtggggctgccgccgagtgtggggctgccgccgagtgtgtggctccgctcctgcccacccagggagggcagcccctgtgccactggcctggccacccgagggagtcagcagggtggctcacaggctcactgagagag

SEQ ID NO: 3 - DNA, 550 bp, synthetic construct
  source 1..550: mol_type = other DNA
gctgagacccacagcctgggcctggatgcaaattcttctctgagactcaggcggttggccaggtgggcaccgggcctctgggatctggatgccaccctccaaggggcctcagatgccagcagcaaggggctgtctgccctcgcaatgcgcctttccagacgcccaaatccttcccatttgaccaccctttgcagccaccactttctcaaagtagatttactttcaatctccatttgctaaatctcttccctctaaaccttttggggatggagggattaagcctgattacagatgttgggggtggtagcaggagtcgggcaggaggggccaccaaaagccagcacatgctcctcctaggctgaaccagcctccggccggcctcgccccaggatctcggccccctcgcccagtgcgtggggctgccgccgagtgtggggctgccgccgagtgtgtggctccgctcctgcccacccagggagggcagcccctgtgccactggcctggccacccgagggagtcagcagggtggctcacaggctcactgagagag

SEQ ID NO: 4 - DNA, 802 bp, synthetic construct
  source 1..802: mol_type = other DNA
tttatagcataaattgtctattctctgcagtgtattttttagccctcctcccccagaaaatgtaattggaaatatcaactcatgttgaatgtgtttgctgtacctgtttatgttttattgattattttctgggagaagtttggagttgtgtttggtttggctctgtgcaacctcatttatttgctctgtaaagctgataagcacaagaagtgaaatgacactcaggcattttaagatgcgagtcatcttcattctgaactaagtgaaaacaaaacagattttctatcaacctaaaatcctcctactgggggcagtagatgtttttagaaaattggctttggctttgattgacaatgtttggaagatgtcctataatttgagagtgtatgtgtgtgtgtctgggtgtgtgtgtgtaaatgctggacctgggaagatggaagccctcagccaggagaataagaggacacaatacccccaagccttccatgacctagagattaaggggatttaacgtcttaaaacctccattaagtagacagtagcaagagacatgttgccctcagtgatatgcaaaggcatatctgatgggtcagtatctgccatcctcctcttttgcaagctctgaggttagactcagccatgggtgaaggaattacagcatccattgggagcaggcagagtccaggaaagagatttttctgttacctcagatgcccatcgcgccaggagcaattttcccagcctcttgtagaaagcacatattagtatctatctcactgcttttcagaaactgtatcttcaa

SEQ ID NO: 5 - DNA, 480 bp, synthetic construct
  source 1..480: mol_type = other DNA
tcccccagaaaatgtaattggaaatatcaactcatgttgaatgtgtttgctgtacctgtttatgttttattgattattttctgggagaagtttggagttgtgtttggtttggctctgtgcaacctcatttatttgctctgtaaagctgataagcacaagaagtgaaatgacactcaggcattttaagatgcgagtcatcttcattctgaactaagtgaaaacaaaacagattttctatcaacctaaaatcctcctactgggggcagtagatgtttttagaaaattggctttggctttgattgacaatgtttggaagatgtcctataatttgagagtgtatgtgtgtgtgtctgggtgtgtgtgtgtaaatgctggacctgggaagatggaagccctcagccaggagaataagaggacacaatacccccaagccttccatgacctagagattaaggggatttaacgtcttaaaacctccat

SEQ ID NO: 6 - DNA, 1251 bp, synthetic construct
  source 1..1251: mol_type = other DNA
tgaaggggggagagcagggattagaagcactcagaaggggctgagagtcatgtggggctcacactgcatttgcagctgggttcaccctgacctcaggcccaacttagatgaggaaggattagcagtaattagtgccatgtgccgccttctcccagctccccggggcacgaacactgcccagctgatgaggggattctgaaagaaccattatgtccaattgtctcaattatgcaaaccctgctgacatttccagccagggaagggcggctgggtgggagggggccatggcggggccacttcaaaggaaaagctctagctcccctacctctctcacatcctaaggctgcctttgtgggattccacacagaacagcctggaagcttggggccctggcttccttttctggcctgggagtcaggtcatggggccatcgcttcacagcaatcatgagggcccaggcccaagtgctcacatgctcctcatggggactgctcctcttaaagggtgggccctcctcacccagctccctgccctggccaaggaggaggctgaaagagcctgagctgtgccctctccattccactgctgtggcaggtaagctcagatgcgggtaagcacaggtgaagggaggtcaggtgcaggtatcctcaggtgtgggtaaactcaagcgtggacaaactcaggtgcagataaccacagatgcagttaagctcaggtgttggtaacctcaggtgcaggtaggctcaggtgcaagtaagagcaggtgcaggcaagctcaggtgtgctttctggggcctgttactcatctcctcttgaggctggctggacaggaccctatggagcagctggtgaacctgtgttcagcctgggttccaagaggctgtctcagcagaagggacccaccaggttgattcacagaggggataagtactctgtcagctggtctcaaagaggctgaaaccctctgagcttccctcagggccagcttctaaatccaggtgccagggatctgctcaggagccccggctccaggcctcaacctcttgcctgtcattccttagcatcttactttgcttcagggaaaaggtgcaccttccttagaaccccagaaaatgctgaagttctaggagagacagggtttatacttgtaagcctttatcagctgatatttcacctgtgaaagccttggggaagagattggttacacggaacaggatcaggaggggagattactgctccctctcactgctg

SEQ ID NO: 7 - DNA, 881 bp, synthetic construct
  source 1..881: mol_type = other DNA
tgtggggctcacactgcatttgcagctgggttcaccctgacctcaggcccaacttagatgaggaaggattagcagtaattagtgccatgtgccgccttctcccagctccccggggcacgaacactgcccagctgatgaggggattctgaaagaaccattatgtccaattgtctcaattatgcaaaccctgctgacatttccagccagggaagggcgagagcctgagctgtgccctctccattccactgctgtggcaggtaagctcagatgcgggtaagcacaggtgaagggaggtcaggtgcaggtatcctcaggtgtgggtaaactcaagcgtggacaaactcaggtgcagataaccacagatgcagttaagctcaggtgttggtaacctcaggtgcaggtaggctcaggtgcaagtaagagcaggtgcaggcaagctcaggtgtgctttctggggcctgttactcatctcctcttgaggctggctggacaggaccctatggagcagctggtgaacctgtgttcagcctgggttccaagaggctgtctcagcagaagggacccaccaggttgattcacagaggggataagtactctgtcagctggtctcaaagaggctgaaaccctctgagcttccctcagggccagcttctaaatccaggtgccagggatctgctcaggagccccggctccaggcctcaacctcttgcctgtcattccttagcatcttactttgcttcagggaaaaggtgcaccttccttagaaccccagaaaatgctgaagttctaggagagacagggtttatacttgtaagcctttatcagctgatatttcacctgtgaaagccttggggaagagattggttacacggaacaggatc

SEQ ID NO: 8 - DNA, 460 bp, synthetic construct
  source 1..460: mol_type = other DNA
tgtggggctcacactgcatttgcagctgggttcaccctgacctcaggcccaacttagatgaggaaggattagcagtaattagtgccatgtgccgccttctcccagctccccggggcacgaacactgcccagctgatgaggggattctgaaagaaccattatggggataagtactctgtcagctggtctcaaagaggctgaaaccctctgagcttccctcagggccagcttctaaatccaggtgccagggatctgctcaggagccccggctccaggcctcaacctcttgcctgtcattccttagcatcttactttgcttcagggaaaaggtgcaccttccttagaaccccagaaaatgctgaagttctaggagagacagggtttatacttgtaagcctttatcagctgatatttcacctgtgaaagccttggggaagagattggttacacggaacaggatc

SEQ ID NO: 9 - DNA, 277 bp, synthetic construct
  source 1..277: mol_type = other DNA
cagaaagttgacaaactacagctgagtatcaggtcggcactggaggcggccaggtgggggcagcagagagctgagtgggcagaaaccggggctcataggcggtgaggttctgtcaacggagctgcaagagaagtaaccctgcagggtcccaccaaatgacccaaagtggaaagggccaggcggcccgggtcccttactggacagatctgcgcagtaagcacaagtcagcactgttgctgtggcactggcaccatcagtacttgacctaggatcacct

SEQ ID NO: 10 - DNA, 622 bp, synthetic construct
  source 1..622: mol_type = other DNA
gagcacttgagctttcagggtgcagggcctgtgggaaacgggccatggacctcctcggggggatggaggcccctcagtcgggaggtgcaagaaagaggagctgcttttggggtcacagaggggccaggggaggcagagcttgtgcccaaccttggggtcaacccggctgccaataggcccatgcaaacccaagacagtgggccatcaggaaggcactgtggaggggtaatccgcgtaatggcccagaacacggcgtaacagctggctgtggctaatgctcctcaatatctgcttttatgtgattaatggctgtggataaaaccttgatcccaggaaagcaggcccagcggctaagcctagccaagagcaccactttggttatgctgggagcccgagtcattttggcgattttcattttaaccaagctgtcattttagtatgtgaggaaaaaaaataaaagtggtaggaactacactcacagagagcccagagagggggcagcaggggggtgggggcgagcctggtgctggaagtgtgaaaacagctgggggcccaagtgccctgactcccctggccacccactcactgcttccacccactctcacttcccttgggttcacac

SEQ ID NO: 11 - DNA, 400 bp, synthetic construct
  source 1..400: mol_type = other DNA
gcaagaaagaggagctgcttttggggtcacagaggggccaggggaggcagagcttgtgcccaaccttggggtcaacccggctgccaataggcccatgcaaacccaagacagtgggccatcaggaaggcactgtggaggggtaatccgcgtaatggcccagaacacggcgtaacagctggctgtggctaatgctcctcaatatctgcttttatgtgattaatggctgtggataaaaccttgatcccaggaaagcaggcccagcggctaagcctagccaagagcaccactttggttatgctgggagcccgagtcattttggcgattttcattttaaccaagctgtcattttagtatgtgaggaaaaaaaataaaagtggtaggaactacactcacagagagc

SEQ ID NO: 12 - DNA, 284 bp, synthetic construct
  source 1..284: mol_type = other DNA
catcaggaaggcactgtggaggggtaatccgcgtaatggcccagaacacggcgtaacagctggctgtggctaatgctcctcaatatctgcttttatgtgattaatggctgtggataaaaccttgatcccaggaaagcaggcccagcggctaagcctagccaagagcaccactttggttatgctgggagcccgagtcattttggcgattttcattttaaccaagctgtcattttagtatgtgaggaaaaaaaataaaagtggtaggaactacactcacagagagc

SEQ ID NO: 13 - DNA, 160 bp, synthetic construct
  source 1..160: mol_type = other DNA
cggggggatggaggcccctcagtcgggaggtgcaagaaagaggagctgcttttggggtcacagaggggccaggggaggcagagcttgtgcccaaccttggggtcagctggctgtggctaatgctcctcaatatctgcttttatgtgattaatggctgtgg

SEQ ID NO: 14 - DNA, 56 bp, synthetic construct
  source 1..56: mol_type = other DNA
agctggctgtggctaatgctcctcaatatctgcttttatgtgattaatggctgtgg

SEQ ID NO: 15 - DNA, 1352 bp, synthetic construct
  source 1..1352: mol_type = other DNA
tttatagcataaattgtctattctctgcagtgtattttttagccctcctcccccagaaaatgtaattggaaatatcaactcatgttgaatgtgtttgctgtacctgtttatgttttattgattattttctgggagaagtttggagttgtgtttggtttggctctgtgcaacctcatttatttgctctgtaaagctgataagcacaagaagtgaaatgacactcaggcattttaagatgcgagtcatcttcattctgaactaagtgaaaacaaaacagattttctatcaacctaaaatcctcctactgggggcagtagatgtttttagaaaattggctttggctttgattgacaatgtttggaagatgtcctataatttgagagtgtatgtgtgtgtgtctgggtgtgtgtgtgtaaatgctggacctgggaagatggaagccctcagccaggagaataagaggacacaatacccccaagccttccatgacctagagattaaggggatttaacgtcttaaaacctccattaagtagacagtagcaagagacatgttgccctcagtgatatgcaaaggcatatctgatgggtcagtatctgccatcctcctcttttgcaagctctgaggttagactcagccatgggtgaaggaattacagcatccattgggagcaggcagagtccaggaaagagatttttctgttacctcagatgcccatcgcgccaggagcaattttcccagcctcttgtagaaagcacatattagtatctatctcactgcttttcagaaactgtatcttcaagctgagacccacagcctgggcctggatgcaaattcttctctgagactcaggcggttggccaggtgggcaccgggcctctgggatctggatgccaccctccaaggggcctcagatgccagcagcaaggggctgtctgccctcgcaatgcgcctttccagacgcccaaatccttcccatttgaccaccctttgcagccaccactttctcaaagtagatttactttcaatctccatttgctaaatctcttccctctaaaccttttggggatggagggattaagcctgattacagatgttgggggtggtagcaggagtcgggcaggaggggccaccaaaagccagcacatgctcctcctaggctgaaccagcctccggccggcctcgccccaggatctcggccccctcgcccagtgcgtggggctgccgccgagtgtggggctgccgccgagtgtgtggctccgctcctgcccacccagggagggcagcccctgtgccactggcctggccacccgagggagtcagcagggtggctcacaggctcactgagagag

SEQ ID NO: 16 - DNA, 1030 bp, synthetic construct
  source 1..1030: mol_type = other DNA
tcccccagaaaatgtaattggaaatatcaactcatgttgaatgtgtttgctgtacctgtttatgttttattgattattttctgggagaagtttggagttgtgtttggtttggctctgtgcaacctcatttatttgctctgtaaagctgataagcacaagaagtgaaatgacactcaggcattttaagatgcgagtcatcttcattctgaactaagtgaaaacaaaacagattttctatcaacctaaaatcctcctactgggggcagtagatgtttttagaaaattggctttggctttgattgacaatgtttggaagatgtcctataatttgagagtgtatgtgtgtgtgtctgggtgtgtgtgtgtaaatgctggacctgggaagatggaagccctcagccaggagaataagaggacacaatacccccaagccttccatgacctagagattaaggggatttaacgtcttaaaacctccatgctgagacccacagcctgggcctggatgcaaattcttctctgagactcaggcggttggccaggtgggcaccgggcctctgggatctggatgccaccctccaaggggcctcagatgccagcagcaaggggctgtctgccctcgcaatgcgcctttccagacgcccaaatccttcccatttgaccaccctttgcagccaccactttctcaaagtagatttactttcaatctccatttgctaaatctcttccctctaaaccttttggggatggagggattaagcctgattacagatgttgggggtggtagcaggagtcgggcaggaggggccaccaaaagccagcacatgctcctcctaggctgaaccagcctccggccggcctcgccccaggatctcggccccctcgcccagtgcgtggggctgccgccgagtgtggggctgccgccgagtgtgtggctccgctcctgcccacccagggagggcagcccctgtgccactggcctggccacccgagggagtcagcagggtggctcacaggctcactgagagag

SEQ ID NO: 17 - DNA, 1801 bp, synthetic construct
  source 1..1801: mol_type = other DNA
tgaaggggggagagcagggattagaagcactcagaaggggctgagagtcatgtggggctcacactgcatttgcagctgggttcaccctgacctcaggcccaacttagatgaggaaggattagcagtaattagtgccatgtgccgccttctcccagctccccggggcacgaacactgcccagctgatgaggggattctgaaagaaccattatgtccaattgtctcaattatgcaaaccctgctgacatttccagccagggaagggcggctgggtgggagggggccatggcggggccacttcaaaggaaaagctctagctcccctacctctctcacatcctaaggctgcctttgtgggattccacacagaacagcctggaagcttggggccctggcttccttttctggcctgggagtcaggtcatggggccatcgcttcacagcaatcatgagggcccaggcccaagtgctcacatgctcctcatggggactgctcctcttaaagggtgggccctcctcacccagctccctgccctggccaaggaggaggctgaaagagcctgagctgtgccctctccattccactgctgtggcaggtaagctcagatgcgggtaagcacaggtgaagggaggtcaggtgcaggtatcctcaggtgtgggtaaactcaagcgtggacaaactcaggtgcagataaccacagatgcagttaagctcaggtgttggtaacctcaggtgcaggtaggctcaggtgcaagtaagagcaggtgcaggcaagctcaggtgtgctttctggggcctgttactcatctcctcttgaggctggctggacaggaccctatggagcagctggtgaacctgtgttcagcctgggttccaagaggctgtctcagcagaagggacccaccaggttgattcacagaggggataagtactctgtcagctggtctcaaagaggctgaaaccctctgagcttccctcagggccagcttctaaatccaggtgccagggatctgctcaggagccccggctccaggcctcaacctcttgcctgtcattccttagcatcttactttgcttcagggaaaaggtgcaccttccttagaaccccagaaaatgctgaagttctaggagagacagggtttatacttgtaagcctttatcagctgatatttcacctgtgaaagccttggggaagagattggttacacggaacaggatcaggaggggagattactgctccctctcactgctggctgagacccacagcctgggcctggatgcaaattcttctctgagactcaggcggttggccaggtgggcaccgggcctctgggatctggatgccaccctccaaggggcctcagatgccagcagcaaggggctgtctgccctcgcaatgcgcctttccagacgcccaaatccttcccatttgaccaccctttgcagccaccactttctcaaagtagatttactttcaatctccatttgctaaatctcttccctctaaaccttttggggatggagggattaagcctgattacagatgttgggggtggtagcaggagtcgggcaggaggggccaccaaaagccagcacatgctcctcctaggctgaaccagcctccggccggcctcgccccaggatctcggccccctcgcccagtgcgtggggctgccgccgagtgtggggctgccgccgagtgtgtggctccgctcctgcccacccagggagggcagcccctgtgccactggcctggccacccgagggagtcagcagggtggctcacaggctcactgagagag

SEQ ID NO: 18 - DNA, 1431 bp, synthetic construct
  source 1..1431: mol_type = other DNA
tgtggggctcacactgcatttgcagctgggttcaccctgacctcaggcccaacttagatgaggaaggattagcagtaattagtgccatgtgccgccttctcccagctccccggggcacgaacactgcccagctgatgaggggattctgaaagaaccattatgtccaattgtctcaattatgcaaaccctgctgacatttccagccagggaagggcgagagcctgagctgtgccctctccattccactgctgtggcaggtaagctcagatgcgggtaagcacaggtgaagggaggtcaggtgcaggtatcctcaggtgtgggtaaactcaagcgtggacaaactcaggtgcagataaccacagatgcagttaagctcaggtgttggtaacctcaggtgcaggtaggctcaggtgcaagtaagagcaggtgcaggcaagctcaggtgtgctttctggggcctgttactcatctcctcttgaggctggctggacaggaccctatggagcagctggtgaacctgtgttcagcctgggttccaagaggctgtctcagcagaagggacccaccaggttgattcacagaggggataagtactctgtcagctggtctcaaagaggctgaaaccctctgagcttccctcagggccagcttctaaatccaggtgccagggatctgctcaggagccccggctccaggcctcaacctcttgcctgtcattccttagcatcttactttgcttcagggaaaaggtgcaccttccttagaaccccagaaaatgctgaagttctaggagagacagggtttatacttgtaagcctttatcagctgatatttcacctgtgaaagccttggggaagagattggttacacggaacaggatcgctgagacccacagcctgggcctggatgcaaattcttctctgagactcaggcggttggccaggtgggcaccgggcctctgggatctggatgccaccctccaaggggcctcagatgccagcagcaaggggctgtctgccctcgcaatgcgcctttccagacgcccaaatccttcccatttgaccaccctttgcagccaccactttctcaaagtagatttactttcaatctccatttgctaaatctcttccctctaaaccttttggggatggagggattaagcctgattacagatgttgggggtggtagcaggagtcgggcaggaggggccaccaaaagccagcacatgctcctcctaggctgaaccagcctccggccggcctcgccccaggatctcggccccctcgcccagtgcgtggggctgccgccgagtgtggggctgccgccgagtgtgtggctccgctcctgcccacccagggagggcagcccctgtgccactggcctggccacccgagggagtcagcagggtggctcacaggctcactgagagag

SEQ ID NO: 19 - DNA, 1010 bp, synthetic construct
  source 1..1010: mol_type = other DNA
tgtggggctcacactgcatttgcagctgggttcaccctgacctcaggcccaacttagatgaggaaggattagcagtaattagtgccatgtgccgccttctcccagctccccggggcacgaacactgcccagctgatgaggggattctgaaagaaccattatggggataagtactctgtcagctggtctcaaagaggctgaaaccctctgagcttccctcagggccagcttctaaatccaggtgccagggatctgctcaggagccccggctccaggcctcaacctcttgcctgtcattccttagcatcttactttgcttcagggaaaaggtgcaccttccttagaaccccagaaaatgctgaagttctaggagagacagggtttatacttgtaagcctttatcagctgatatttcacctgtgaaagccttggggaagagattggttacacggaacaggatcgctgagacccacagcctgggcctggatgcaaattcttctctgagactcaggcggttggccaggtgggcaccgggcctctgggatctggatgccaccctccaaggggcctcagatgccagcagcaaggggctgtctgccctcgcaatgcgcctttccagacgcccaaatccttcccatttgaccaccctttgcagccaccactttctcaaagtagatttactttcaatctccatttgctaaatctcttccctctaaaccttttggggatggagggattaagcctgattacagatgttgggggtggtagcaggagtcgggcaggaggggccaccaaaagccagcacatgctcctcctaggctgaaccagcctccggccggcctcgccccaggatctcggccccctcgcccagtgcgtggggctgccgccgagtgtggggctgccgccgagtgtgtggctccgctcctgcccacccagggagggcagcccctgtgccactggcctggccacccgagggagtcagcagggtggctcacaggctcactgagagag

SEQ ID NO: 20 - DNA, 827 bp, synthetic construct
  source 1..827: mol_type = other DNA
cagaaagttgacaaactacagctgagtatcaggtcggcactggaggcggccaggtgggggcagcagagagctgagtgggcagaaaccggggctcataggcggtgaggttctgtcaacggagctgcaagagaagtaaccctgcagggtcccaccaaatgacccaaagtggaaagggccaggcggcccgggtcccttactggacagatctgcgcagtaagcacaagtcagcactgttgctgtggcactggcaccatcagtacttgacctaggatcacctgctgagacccacagcctgggcctggatgcaaattcttctctgagactcaggcggttggccaggtgggcaccgggcctctgggatctggatgccaccctccaaggggcctcagatgccagcagcaaggggctgtctgccctcgcaatgcgcctttccagacgcccaaatccttcccatttgaccaccctttgcagccaccactttctcaaagtagatttactttcaatctccatttgctaaatctcttccctctaaaccttttggggatggagggattaagcctgattacagatgttgggggtggtagcaggagtcgggcaggaggggccaccaaaagccagcacatgctcctcctaggctgaaccagcctccggccggcctcgccccaggatctcggccccctcgcccagtgcgtggggctgccgccgagtgtggggctgccgccgagtgtgtggctccgctcctgcccacccagggagggcagcccctgtgccactggcctggccacccgagggagtcagcagggtggctcacaggctcactgagagag

SEQ ID NO: 21 - DNA, 1172 bp, synthetic construct
  source 1..1172: mol_type = other DNA
gagcacttgagctttcagggtgcagggcctgtgggaaacgggccatggacctcctcggggggatggaggcccctcagtcgggaggtgcaagaaagaggagctgcttttggggtcacagaggggccaggggaggcagagcttgtgcccaaccttggggtcaacccggctgccaataggcccatgcaaacccaagacagtgggccatcaggaaggcactgtggaggggtaatccgcgtaatggcccagaacacggcgtaacagctggctgtggctaatgctcctcaatatctgcttttatgtgattaatggctgtggataaaaccttgatcccaggaaagcaggcccagcggctaagcctagccaagagcaccactttggttatgctgggagcccgagtcattttggcgattttcattttaaccaagctgtcattttagtatgtgaggaaaaaaaataaaagtggtaggaactacactcacagagagcccagagagggggcagcaggggggtgggggcgagcctggtgctggaagtgtgaaaacagctgggggcccaagtgccctgactcccctggccacccactcactgcttccacccactctcacttcccttgggttcacacgctgagacccacagcctgggcctggatgcaaattcttctctgagactcaggcggttggccaggtgggcaccgggcctctgggatctggatgccaccctccaaggggcctcagatgccagcagcaaggggctgtctgccctcgcaatgcgcctttccagacgcccaaatccttcccatttgaccaccctttgcagccaccactttctcaaagtagatttactttcaatctccatttgctaaatctcttccctctaaaccttttggggatggagggattaagcctgattacagatgttgggggtggtagcaggagtcgggcaggaggggccaccaaaagccagcacatgctcctcctaggctgaaccagcctccggccggcctcgccccaggatctcggccccctcgcccagtgcgtggggctgccgccgagtgtggggctgccgccgagtgtgtggctccgctcctgcccacccagggagggcagcccctgtgccactggcctggccacccgagggagtcagcagggtggctcacaggctcactgagagag

SEQ ID NO: 22 - DNA, 950 bp, synthetic construct
  source 1..950: mol_type = other DNA
gcaagaaagaggagctgcttttggggtcacagaggggccaggggaggcagagcttgtgcccaaccttggggtcaacccggctgccaataggcccatgcaaacccaagacagtgggccatcaggaaggcactgtggaggggtaatccgcgtaatggcccagaacacggcgtaacagctggctgtggctaatgctcctcaatatctgcttttatgtgattaatggctgtggataaaaccttgatcccaggaaagcaggcccagcggctaagcctagccaagagcaccactttggttatgctgggagcccgagtcattttggcgattttcattttaaccaagctgtcattttagtatgtgaggaaaaaaaataaaagtggtaggaactacactcacagagagcgctgagacccacagcctgggcctggatgcaaattcttctctgagactcaggcggttggccaggtgggcaccgggcctctgggatctggatgccaccctccaaggggcctcagatgccagcagcaaggggctgtctgccctcgcaatgcgcctttccagacgcccaaatccttcccatttgaccaccctttgcagccaccactttctcaaagtagatttactttcaatctccatttgctaaatctcttccctctaaaccttttggggatggagggattaagcctgattacagatgttgggggtggtagcaggagtcgggcaggaggggccaccaaaagccagcacatgctcctcctaggctgaaccagcctccggccggcctcgccccaggatctcggccccctcgcccagtgcgtggggctgccgccgagtgtggggctgccgccgagtgtgtggctccgctcctgcccacccagggagggcagcccctgtgccactggcctggccacccgagggagtcagcagggtggctcacaggctcactgagagag

SEQ ID NO: 23 - DNA, 834 bp, synthetic construct
  source 1..834: mol_type = other DNA
catcaggaaggcactgtggaggggtaatccgcgtaatggcccagaacacggcgtaacagctggctgtggctaatgctcctcaatatctgcttttatgtgattaatggctgtggataaaaccttgatcccaggaaagcaggcccagcggctaagcctagccaagagcaccactttggttatgctgggagcccgagtcattttggcgattttcattttaaccaagctgtcattttagtatgtgaggaaaaaaaataaaagtggtaggaactacactcacagagagcgctgagacccacagcctgggcctggatgcaaattcttctctgagactcaggcggttggccaggtgggcaccgggcctctgggatctggatgccaccctccaaggggcctcagatgccagcagcaaggggctgtctgccctcgcaatgcgcctttccagacgcccaaatccttcccatttgaccaccctttgcagccaccactttctcaaagtagatttactttcaatctccatttgctaaatctcttccctctaaaccttttggggatggagggattaagcctgattacagatgttgggggtggtagcaggagtcgggcaggaggggccaccaaaagccagcacatgctcctcctaggctgaaccagcctccggccggcctcgccccaggatctcggccccctcgcccagtgcgtggggctgccgccgagtgtggggctgccgccgagtgtgtggctccgctcctgcccacccagggagggcagcccctgtgccactggcctggccacccgagggagtcagcagggtggctcacaggctcactgagagag

SEQ ID NO: 24 - DNA, 710 bp, synthetic construct
  source 1..710: mol_type = other DNA
cggggggatggaggcccctcagtcgggaggtgcaagaaagaggagctgcttttggggtcacagaggggccaggggaggcagagcttgtgcccaaccttggggtcagctggctgtggctaatgctcctcaatatctgcttttatgtgattaatggctgtgggctgagacccacagcctgggcctggatgcaaattcttctctgagactcaggcggttggccaggtgggcaccgggcctctgggatctggatgccaccctccaaggggcctcagatgccagcagcaaggggctgtctgccctcgcaatgcgcctttccagacgcccaaatccttcccatttgaccaccctttgcagccaccactttctcaaagtagatttactttcaatctccatttgctaaatctcttccctctaaaccttttggggatggagggattaagcctgattacagatgttgggggtggtagcaggagtcgggcaggaggggccaccaaaagccagcacatgctcctcctaggctgaaccagcctccggccggcctcgccccaggatctcggccccctcgcccagtgcgtggggctgccgccgagtgtggggctgccgccgagtgtgtggctccgctcctgcccacccagggagggcagcccctgtgccactggcctggccacccgagggagtcagcagggtggctcacaggctcactgagagag

SEQ ID NO: 25 - DNA, 606 bp, synthetic construct
  source 1..606: mol_type = other DNA
agctggctgtggctaatgctcctcaatatctgcttttatgtgattaatggctgtgggctgagacccacagcctgggcctggatgcaaattcttctctgagactcaggcggttggccaggtgggcaccgggcctctgggatctggatgccaccctccaaggggcctcagatgccagcagcaaggggctgtctgccctcgcaatgcgcctttccagacgcccaaatccttcccatttgaccaccctttgcagccaccactttctcaaagtagatttactttcaatctccatttgctaaatctcttccctctaaaccttttggggatggagggattaagcctgattacagatgttgggggtggtagcaggagtcgggcaggaggggccaccaaaagccagcacatgctcctcctaggctgaaccagcctccggccggcctcgccccaggatctcggccccctcgcccagtgcgtggggctgccgccgagtgtggggctgccgccgagtgtgtggctccgctcctgcccacccagggagggcagcccctgtgccactggcctggccacccgagggagtcagcagggtggctcacaggctcactgagagag

SEQ ID NO: 26 - DNA, 1318 bp, synthetic construct
  source 1..1318: mol_type = other DNA
catcaggaaggcactgtggaggggtaatccgcgtaatggcccagaacacggcgtaacagctggctgtggctaatgctcctcaatatctgcttttatgtgattaatggctgtggataaaaccttgatcccaggaaagcaggcccagcggctaagcctagccaagagcaccactttggttatgctgggagcccgagtcattttggcgattttcattttaaccaagctgtcattttagtatgtgaggaaaaaaaataaaagtggtaggaactacactcacagagagccatcaggaaggcactgtggaggggtaatccgcgtaatggcccagaacacggcgtaacagctggctgtggctaatgctcctcaatatctgcttttatgtgattaatggctgtggataaaaccttgatcccaggaaagcaggcccagcggctaagcctagccaagagcaccactttggttatgctgggagcccgagtcattttggcgattttcattttaaccaagctgtcattttagtatgtgaggaaaaaaaataaaagtggtaggaactacactcacagagagcgctgcaaagacccatgaccccatctgcctttaagaggggcaagacaggcacccctgaaatcagaaatgacacagagagccccacacacagagcagcacagaacagacgggccaccggccacaggatcttcagaagaaggcttgctgtgtcgctgccagattaacggggcgaaaatgcgcactggcagctccaaggagagagctgagacccacagcctgggcctggatgcaaattcttctctgagactcaggcggttggccaggtgggcaccgggcctctgggatctggatgccaccctccaaggggcctcagatgccagcagcaaggggctgtctgccctcgcaatgcgcctttccagacgcccaaatccttcccatttgaccaccctttgcagccaccactttctcaaagtagatttactttcaatctccatttgctaaatctcttccctctaaaccttttggggatggagggattaagcctgattacagatgttgggggtggtagcaggagtcgggcaggaggggccaccaaaagccagcacatgctcctcctaggctgaaccagcctccggccggcctcgccccaggatctcggccccctcgcccagtgcgtggggctgccgccgagtgtggggctgccgccgagtgtgtggctccgctcctgcccacccagggagggcagcccctgtgccactggcctggccacccgagggagtcagcagggtggctcacaggctcactgagagag

SEQ ID NO: 27 - DNA, 1150 bp, synthetic construct
  source 1..1150: mol_type = other DNA
gcaagaaagaggagctgcttttggggtcacagaggggccaggggaggcagagcttgtgcccaaccttggggtcaacccggctgccaataggcccatgcaaacccaagacagtgggccatcaggaaggcactgtggaggggtaatccgcgtaatggcccagaacacggcgtaacagctggctgtggctaatgctcctcaatatctgcttttatgtgattaatggctgtggataaaaccttgatcccaggaaagcaggcccagcggctaagcctagccaagagcaccactttggttatgctgggagcccgagtcattttggcgattttcattttaaccaagctgtcattttagtatgtgaggaaaaaaaataaaagtggtaggaactacactcacagagagcgctgcaaagacccatgaccccatctgcctttaagaggggcaagacaggcacccctgaaatcagaaatgacacagagagccccacacacagagcagcacagaacagacgggccaccggccacaggatcttcagaagaaggcttgctgtgtcgctgccagattaacggggcgaaaatgcgcactggcagctccaaggagagagctgagacccacagcctgggcctggatgcaaattcttctctgagactcaggcggttggccaggtgggcaccgggcctctgggatctggatgccaccctccaaggggcctcagatgccagcagcaaggggctgtctgccctcgcaatgcgcctttccagacgcccaaatccttcccatttgaccaccctttgcagccaccactttctcaaagtagatttactttcaatctccatttgctaaatctcttccctctaaaccttttggggatggagggattaagcctgattacagatgttgggggtggtagcaggagtcgggcaggaggggccaccaaaagccagcacatgctcctcctaggctgaaccagcctccggccggcctcgccccaggatctcggccccctcgcccagtgcgtggggctgccgccgagtgtggggctgccgccgagtgtgtggctccgctcctgcccacccagggagggcagcccctgtgccactggcctggccacccgagggagtcagcagggtggctcacaggctcactgagagag

SEQ ID NO: 28 - DNA, 910 bp, synthetic construct
  source 1..910: mol_type = other DNA
cggggggatggaggcccctcagtcgggaggtgcaagaaagaggagctgcttttggggtcacagaggggccaggggaggcagagcttgtgcccaaccttggggtcagctggctgtggctaatgctcctcaatatctgcttttatgtgattaatggctgtgggctgcaaagacccatgaccccatctgcctttaagaggggcaagacaggcacccctgaaatcagaaatgacacagagagccccacacacagagcagcacagaacagacgggccaccggccacaggatcttcagaagaaggcttgctgtgtcgctgccagattaacggggcgaaaatgcgcactggcagctccaaggagagagctgagacccacagcctgggcctggatgcaaattcttctctgagactcaggcggttggccaggtgggcaccgggcctctgggatctggatgccaccctccaaggggcctcagatgccagcagcaaggggctgtctgccctcgcaatgcgcctttccagacgcccaaatccttcccatttgaccaccctttgcagccaccactttctcaaagtagatttactttcaatctccatttgctaaatctcttccctctaaaccttttggggatggagggattaagcctgattacagatgttgggggtggtagcaggagtcgggcaggaggggccaccaaaagccagcacatgctcctcctaggctgaaccagcctccggccggcctcgccccaggatctcggccccctcgcccagtgcgtggggctgccgccgagtgtggggctgccgccgagtgtgtggctccgctcctgcccacccagggagggcagcccctgtgccactggcctggccacccgagggagtcagcagggtggctcacaggctcactgagagag

SEQ ID NO: 29 - DNA, 1390 bp, synthetic construct
  source 1..1390: mol_type = other DNA
tcccccagaaaatgtaattggaaatatcaactcatgttgaatgtgtttgctgtacctgtttatgttttattgattattttctgggagaagtttggagttgtgtttggtttggctctgtgcaacctcatttatttgctctgtaaagctgataagcacaagaagtgaaatgacactcaggcattttaagatgcgagtcatcttcattctgaactaagtgaaaacaaaacagattttctatcaacctaaaatcctcctactgggggcagtagatgtttttagaaaattggctttggctttgattgacaatgtttggaagatgtcctataatttgagagtgtatgtgtgtgtgtctgggtgtgtgtgtgtaaatgctggacctgggaagatggaagccctcagccaggagaataagaggacacaatacccccaagccttccatgacctagagattaaggggatttaacgtcttaaaacctccatcggggggatggaggcccctcagtcgggaggtgcaagaaagaggagctgcttttggggtcacagaggggccaggggaggcagagcttgtgcccaaccttggggtcagctggctgtggctaatgctcctcaatatctgcttttatgtgattaatggctgtgggctgcaaagacccatgaccccatctgcctttaagaggggcaagacaggcacccctgaaatcagaaatgacacagagagccccacacacagagcagcacagaacagacgggccaccggccacaggatcttcagaagaaggcttgctgtgtcgctgccagattaacggggcgaaaatgcgcactggcagctccaaggagagagctgagacccacagcctgggcctggatgcaaattcttctctgagactcaggcggttggccaggtgggcaccgggcctctgggatctggatgccaccctccaaggggcctcagatgccagcagcaaggggctgtctgccctcgcaatgcgcctttccagacgcccaaatccttcccatttgaccaccctttgcagccaccactttctcaaagtagatttactttcaatctccatttgctaaatctcttccctctaaaccttttggggatggagggattaagcctgattacagatgttgggggtggtagcaggagtcgggcaggaggggccaccaaaagccagcacatgctcctcctaggctgaaccagcctccggccggcctcgccccaggatctcggccccctcgcccagtgcgtggggctgccgccgagtgtggggctgccgccgagtgtgtggctccgctcctgcccacccagggagggcagcccctgtgccactggcctggccacccgagggagtcagcagggtggctcacaggctcactgagagag

SEQ ID NO: 30 - DNA, 1370 bp, synthetic construct
  source 1..1370: mol_type = other DNA
tgtggggctcacactgcatttgcagctgggttcaccctgacctcaggcccaacttagatgaggaaggattagcagtaattagtgccatgtgccgccttctcccagctccccggggcacgaacactgcccagctgatgaggggattctgaaagaaccattatggggataagtactctgtcagctggtctcaaagaggctgaaaccctctgagcttccctcagggccagcttctaaatccaggtgccagggatctgctcaggagccccggctccaggcctcaacctcttgcctgtcattccttagcatcttactttgcttcagggaaaaggtgcaccttccttagaaccccagaaaatgctgaagttctaggagagacagggtttatacttgtaagcctttatcagctgatatttcacctgtgaaagccttggggaagagattggttacacggaacaggatccggggggatggaggcccctcagtcgggaggtgcaagaaagaggagctgcttttggggtcacagaggggccaggggaggcagagcttgtgcccaaccttggggtcagctggctgtggctaatgctcctcaatatctgcttttatgtgattaatggctgtgggctgcaaagacccatgaccccatctgcctttaagaggggcaagacaggcacccctgaaatcagaaatgacacagagagccccacacacagagcagcacagaacagacgggccaccggccacaggatcttcagaagaaggcttgctgtgtcgctgccagattaacggggcgaaaatgcgcactggcagctccaaggagagagctgagacccacagcctgggcctggatgcaaattcttctctgagactcaggcggttggccaggtgggcaccgggcctctgggatctggatgccaccctccaaggggcctcagatgccagcagcaaggggctgtctgccctcgcaatgcgcctttccagacgcccaaatccttcccatttgaccaccctttgcagccaccactttctcaaagtagatttactttcaatctccatttgctaaatctcttccctctaaaccttttggggatggagggattaagcctgattacagatgttgggggtggtagcaggagtcgggcaggaggggccaccaaaagccagcacatgctcctcctaggctgaaccagcctccggccggcctcgccccaggatctcggccccctcgcccagtgcgtggggctgccgccgagtgtggggctgccgccgagtgtgtggctccgctcctgcccacccagggagggcagcccctgtgccactggcctggccacccgagggagtcagcagggtggctcacaggctcactgagagag

SEQ ID NO: 31 - DNA, 1683 bp, synthetic construct
  source 1..1683: mol_type = other DNA
gagcacttgagctttcagggtgcagggcctgtgggaaacgggccatggacctcctcggggggatggaggcccctcagtcgggaggtgcaagaaagaggagctgcttttggggtcacagaggggccaggggaggcagagcttgtgcccaaccttggggtcaacccggctgccaataggcccatgcaaacccaagacagtgggccatcaggaaggcactgtggaggggtaatccgcgtaatggcccagaacacggcgtaacagctggctgtggctaatgctcctcaatatctgcttttatgtgattaatggctgtggataaaaccttgatcccaggaaagcaggcccagcggctaagcctagccaagagcaccactttggttatgctgggagcccgagtcattttggcgattttcattttaaccaagctgtcattttagtatgtgaggaaaaaaaataaaagtggtaggaactacactcacagagagcccagagagggggcagcaggggggtgggggcgagcctggtgctggaagtgtgaaaacagctgggggcccaagtgccctgactcccctggccacccactcactgcttccacccactctcacttcccttgggttcacactgtgttggttgtaagccagaccccaagaggtggaggtcatgcctccaccctccaaacttccacagccgacaggcctcccagaggaggtggtgggtcctggcctcacagctatgagggctccacagccttctattattttattttcagcttgctggtccttagataaaaatctatctaagacgatgggaatacatggcctgttctctctgagctccagtctgttcccttgcatgtgggaggtgacatgcatgtgcctgtaagagacagaggagggtcggcagcaagggtggtacacttcaggccaggcttgtgctgcaaagacccatgaccccatctgcctttaagaggggcaagacaggcacccctgaaatcagaaatgacacagagagccccacacacagagcagcacagaacagacgggccaccggccacaggatcttcagaagaaggcttgctgtgtcgctgccagattaacggggcgaaaatgcgcactggcagctccaaggagagagctgagacccacagcctgggcctggatgcaaattcttctctgagactcaggcggttggccaggtgggcaccgggcctctgggatctggatgccaccctccaaggggcctcagatgccagcagcaaggggctgtctgccctcgcaatgcgcctttccagacgcccaaatccttcccatttgaccaccctttgcagccaccactttctcaaagtagatttactttcaatctccatttgctaaatctcttccctctaaaccttttggggatggagggattaagcctgattacagatgttgggggtggtagcaggagtcgggcaggaggggccaccaaaagccagcacatgctcctcctaggctgaaccagcctccggccggcctcgccccaggatctcggccccctcgcccagtgcgtggggctgccgccgagtgtggggctgccgccgagtgtgtggctccgctcctgcccacccagggagggcagcccctgtgccactggcctggccacccgagggagtcagcagggtggctcacaggctcactgagagag

SEQ ID NO: 32 - DNA, 1243 bp, synthetic construct
  source 1..1243: mol_type = other DNA
gggtctccaacttgccaactgtagatcttggaacctttcatccttcataactgcataagccaattccttctaataaatctgtataatatatctgtctatataataaatatgtacttacataactctgtatgttacatctatctattctatctatctatctatctatctatctatctatctatctatcatctatctatctatttatctattctctgtgtctttggagaaccctgacatagtaagcaatcatatcacctgcaaatgatgaaagctgtgtattttccaaatcagtcgttttatgtctttttttcttgcactgactagtgccccctagagggaatgataattggaattattgtcttgctctgattttaaaggaagtagatacttcaaataattcatcatggagtgcaatattttctgtaggcttttagtagataacttcatcagtttaaagaagatccttagattatgaaacatttacaattatgaatgaatattagatgttatcaaatgctttttctgcatccatttagataatcatgtttttcctttaatctgttaatgcggtgaattacattaatagatttcctaagtcattaatctgctaaagtgcatttctgggacaaaccagacttggttatgacattgtatgtatttcagtttgcaaatattggactaggatttttgtatctatattccttagtttgacctgtaaattttatttcttgtactaagtattagcctcacgaaaggcattgtcaaatgttcaattgatataatgctagcggaggggtctccaccctcggagcggtctctcatccctccctagaatccttaaatcctctctcgctcagggcctcggccgcatctgtcacagacttgtcctgaaccgacagcggctggcgcaggtgactggcttggggcgggagcctgggtgtgcgctggggatggaccccgaggaagaggggccaagctgtcgggaagcggcagggctggaggggtggaggcagtggtcgggcgggaccccgggcgacagggttcggcgcttgtaagagcgagacggaggcccgggcaggccggctgagctaactccccagagccgaagtggaaggcgcgccccgagcgccttctccccaggaccccggtgtccctccccgcgccccgagcccgcgctctccttcccccgccctcagagcgctccccgcccctctgtctccccgcagcccgctagacgagccga

SEQ ID NO: 33 - DNA, 1488 bp, synthetic construct
  source 1..1488: mol_type = other DNA
tgtgctgggaagatcctcttcctagtcttctaagccagacttctaaaggctgtggctctaccttctgaacccccacagccaagcagttctcttggggcaagaagccacacccagggaggagaaagttggatcttgggttacatggttggcaagttagcttttacttacctctagccttgtctgtctgtattgtgtgctcattttctttttctatgccagtggggctccttctctatgttctgtgagccttgttttttctcctctgtacattagctgatacaaacacccaaggaagtcatcttgagagggtgacacataggtgcactagaatagacctaggagaactgctggattgatttgctgtgtaccactacccttcccctattccacacagcagcagagaagacctgtgtcctgtcctagtctgtgtttttaagagggaagaccatacccctgaaatatgatggacagatccctcacgtggaacacagaatggatctgagatggacacggggcacacacaacaaggtatactgttttgttacccagttcatgggagaaagcatccccattggcttctaggagggagcttccatctacccagtctaggcctaaaaactcagcctactgatatatgaatgccatgggaagctggcctcagtctttgccagtcagattttgtcaacttgacacaagtgttatttgggaagagaaacctcagttgagaaattacctccctcaggttgcctgtaggcaagtctgtagggtgttttcatgactattgattgatgtgggcaagctcagcccacagtagtgtttgtggagtcacacttgggggcaggtggtcctggggtgtataagaaagcaggatgagcaagctatgagcaaccaagcctgtaagcagcatccctccatggcttctgtacctctatggcttgagtacctgccctgacttccctcagtgatgacctgagagtggtaagttgaaataaaccatttctttcccaacctgcttttcatcatggtattttatctgcaccatagaaacattaagacatagcccaacaaggggccttgggcaccagtgctgaaggttctcacatttcaccttgctggatccccaaatcctcatcatgtgcccaccccaaaccctctgcagtcaccactttctcaaagtagattttacttccaattgccatttgctaaatctgcctcctaaaaaccttgcggggggagtagggattaaggctgattacagatgttacagaagctatgtagtctctgagcactgggtgggagtccagccggagggtgagaagcagtccagctccttctgagctgactgagccatcaatatcatctcaaactctgagccctgctgtccagtctcataaagaggactctcttacctcagctgaccagggcctcccatgcagcaggctggacctcacagggaatgcagaagcacccatggggtccatgaggaag

SEQ ID NO: 34 - DNA, 528 bp, synthetic construct
  source 1..528: mol_type = other DNA
agtgatgacctgagagtggtaagttgaaataaaccatttctttcccaacctgcttttcatcatggtattttatctgcaccatagaaacattaagacatagcccaacaaggggccttgggcaccagtgctgaaggttctcacatttcaccttgctggatccccaaatcctcatcatgtgcccaccccaaaccctctgcagtcaccactttctcaaagtagattttacttccaattgccatttgctaaatctgcctcctaaaaaccttgcggggggagtagggattaaggctgattacagatgttacagaagctatgtagtctctgagcactgggtgggagtccagccggagggtgagaagcagtccagctccttctgagctgactgagccatcaatatcatctcaaactctgagccctgctgtccagtctcataaagaggactctcttacctcagctgaccagggcctcccatgcagcaggctggacctcacagggaatgcagaagcacccatggggtccatgaggaag

SEQ ID NO: 35 - DNA, 984 bp, synthetic construct
  source 1..984: mol_type = other DNA
tttctgatcagaactgaggcctctttcaggggagggaactcatgcctggtactgcacaaccgctcaaaagccaatgactcaggtagtcagagggcccaaggggaacctactgctgttgttttgctaaatgaacacgttaaactgccttatatttatgtttgtactcgtagatcaatgctgccttccatcttgaccagagaagccactttctgctggggcagcaatatagactcataactgctccgggtgctgagaataagagattttgagattgccccgccctgactgggacatccctgctgaaatggaaagaactagaactgatttgtctagcatggcagaaacatggctgagcccttgcgtatggtctcagctgagatatactgaggacagggtaaaccaccacacagccattcaccatggtcaggtgtgccccagagtctgcaagatttcaaaaacccgagaatcctgacatgaagtatctcataaataagcttttaggtgttgacatgtttattgagttcaaaacctatagaattgaagttgacttcatttattcattttttgtaagtggcattaatcatagtggcagtccatagctgaacctgctctccccccccccccccccccgcttgagacagtctcaccatgtagtttagatgatcatgaaccctgacccagcctttcaagttttggcattgcaggtgtgtgcaaacaccaggcaggctattctttctaactgagtttttagacattgaattcctttaggttgcagaagatattggtgaatagggatccacttactcctagctggggacttccagtttctagatccaggcccagactctaacttcaatttctctctctctctctctctctctctctctctctctctctctctctctctctctctctctctctccatttgtctctttctctctgtctctgctctgtttctatctctatctctctgtgtgtctccag

SEQ ID NO: 36 - DNA, 664 bp, synthetic construct
  source 1..664: mol_type = other DNA
aaccgctcaaaagccaatgactcaggtagtcagagggcccaaggggaacctactgctgttgttttgctaaatgaacacgttaaactgccttatatttatgtttgtactcgtagatcaatgctgccttccatcttgaccagagaagccactttctgctggggcagcaatatagactcataactgctccgggtgctgagaataagagattttgagattgccccgccctgactgggacatccctgctgaaatggaaagaactagaactgatttgtctagcatggcagaaacatggctgagcccttgcgtatggtctcagctgagatatactgaggacagggtaaaccaccacacagccattcaccatggtcaggtgtgccccagagtctgcaagatttcaaaaacccgagaatcctgacatgaagtatctcataaataagcttttaggtgttgacatgtttattgagttcaaaacctatagaattgaagttgacttcatttattcattttttgtaagtggcattaatcatagtggcagtccatagctgaacctgctctccccccccccccccccccgcttgagacagtctcaccatgtagtttagatgatcatgaaccctgacccagcctttcaagttttggcattgcaggtgtgtgcaaacaccag

SEQ ID NO: 37 - DNA, 1187 bp, synthetic construct
  source 1..1187: mol_type = other DNA
agatactagaagagggagatgctgcccagctctgaagctggggtttcccagcaaatcccaggcatgcgcatggagaagctttgcccagggaagctcagagtatcgagccagttctcaaccctacagaccttcttctctgccaatcaaccagtcaggcctctgggaacccaggctcagtctggatctagtacccagtcccagaaggccctgaagccacgtttgcagagaggagcaaggggctgaaagagccaaactctgtcactgaacttacctgcctcagctgctgagcaagcgggaagggtgcagcctagcctccttcagcctcctcctgggcccaggcaggaagctgaatgaggggggctcactctttaagaggagcagcccacatgaagagcatgtgggtgcctatgcccggtcctcatgatccccgtgagacagaggcagcctcgtgacctggctcccaggctgctcagcgtggtatgcacaaaagccacctccctttgaagtggtccccacctcccctgccccagccaggcctttcagtgctgcaaatgtcagcccactttgcataattgagacaattgggcataatcattctttcagaagcccccactggcaggcagcttatgccccagccctcatgagccaggaagaggagccacgtgcttccaattactgcggagcctttttaagttggtcagagttgggccagaggttgcgacgactccgacggcaaacgctgggtgagtcccacatgactttcaggcccacgtgaagcttctgatcccattctgtttccactccaccagcaatctgcctgactggggtcacagtggccaccacagtgagagctttgtggatttgctgtaccaacacacctgcatgtgtcctagcctctggcatgctttctctgcctgctagaaggaaagtccagaaaggccccttgatatgtatccctttggacttttcttcagcacaggtggtagtgggggctcctgggagcagacccctctctgctttactaggggcttgtatacctgtagatgggtgggatgcctggacaggttcccatctgcacaaggggacaccgagggtagggagtggctgacttgcccagagagtgtgggaaccggagcaggcccggctgcacactttaggatgttctgttcactatagagccctgagga

SEQ ID NO: 38 - DNA, 542 bp, synthetic construct
  source 1..542: mol_type = other DNA
gaaggccctgaagccacgtttgcagagaggagcaaggggctgaaagagccaaactctgtcactgaacttacctgcctcagctgctgagcaagcgggaagggtgcagcctagcctccttcagcctcctcctgggcccaggcaggaagctgaatgaggggggctcactctttaagaggagcagcccacatgaagagcatgtgggtgcctatgcccggtcctcatgatccccgtgagacagaggcagcctcgtgacctggctcccaggctgctcagcgtggtatgcacaaaagccacctccctttgaagtggtccccacctcccctgccccagccaggcctttcagtgctgcaaatgtcagcccactttgcataattgagacaattgggcataatcattctttcagaagcccccactggcaggcagcttatgccccagccctcatgagccaggaagaggagccacgtgcttccaattactgcggagcctttttaagttggtcagagttgggccagaggttgcgacgactccgacggcaaacgctg

SEQ ID NO: 39 - DNA, 876 bp, synthetic construct
  source 1..876: mol_type = other DNA
atctaagccccagggatgtggagttggggccagtgagctaggttcctaggagtaagaaccctttgtccctggctgcttttacatcttcgacaccaggcttggctcccccgtctccccttgtctctctgagctgcccatgagctccattctcacctcttcacggaaatgactcctgactcccagcatcacaaagtgatgggagctgggttcatcggcagggcctgcttttccgggatcaaagtcttatcgacagcctttaatcacatgaaagcagatattcccagggcattaggccccaccagatgctgtgcgcctgcctgggccattaggagattatgcttggacccagccagcactcggcacccatggcttggggatgtgggactcttgatcgttaagccgaggacccagcactctgggtacctgtgctttctcctgccctctctgtaatggcccctagacttctttgcttaggaatctcctctccccaagcagatgtgatgatcccttcgcatggctctgctgacctcagagcacatcctcctggcttgatgctcagtcatgctggcagcctggtaaagcagggaacctaccttcccccatgggctggaggctctgtaggcccaaggcaagtgggtgtccctgtaggtgccagagtagaaaaggctgagcccgaatctggaggaacaggtattcagcaggtaccagggctatggagaattgaaaaggccttggaggccagaagccatagcacatgtcactctgcatggtgagctgaccactcaaagcagacttaacctaggatgcaccactgtccagcctaacgtgacctcatggcaggggctttattctatatttctatgtatatttcatata

SEQ ID NO: 40 - DNA, 1146 bp, synthetic construct
  source 1..1146: mol_type = other DNA
aaccgctcaaaagccaatgactcaggtagtcagagggcccaaggggaacctactgctgttgttttgctaaatgaacacgttaaactgccttatatttatgtttgtactcgtagatcaatgctgccttccatcttgaccagagaagccactttctgctggggcagcaatatagactcataactgctccgggtgctgagaataagagattttgagattgccccgccctgactgggacatccctgctgaaatggaaagaactagaactgatttgtctagcatggcagaaacatggctgagcccttgcgtatggtctcagctgagatatactgaggacagggtaaaccaccacacagccattcaccatggtcaggtgtgccccagagtctgcaagatttcaaaaacccgagaatcctgacatgaagtatctcataaataagcttttaggtgttgacatgtttattgagttcaaaacctatagaattgaagttgacttcatttattcattttttgtaagtggcattaatcatagtggcagtccatagctgaacctgctctccccccccccccccccccgcttgagacagtctcaccatgtagtttagatgatcatgaaccctgagtgatgacctgagagtggtaagttgaaataaaccatttctttcccaacctgcttttcatcatggtattttatctgcaccatagaaacattaagacatagcccaacaaggggccttgggcaccagtgctgaaggttctcacatttcaccttgctggatccccaaatcctcatcatgtgcccaccccaaaccctctgcagtcaccactttctcaaagtagattttacttccaattgccatttgctaaatctgcctcctaaaaaccttgcggggggagtagggattaaggctgattacagatgttacagaagctatgtagtctctgagcactgggtgggagtccagccggagggtgagaagcagtccagctccttctgagctgactgagccatcaatatcatctcaaactctgagccctgctgtccagtctcataaagaggactctcttacctcagctgaccagggcctcccatgcagcaggctggacctcacagggaatgcagaagcacccatggggtccatgaggaag

SEQ ID NO: 41 - DNA, 1070 bp, synthetic construct
  source 1..1070: mol_type = other DNA
gaaggccctgaagccacgtttgcagagaggagcaaggggctgaaagagccaaactctgtcactgaacttacctgcctcagctgctgagcaagcgggaagggtgcagcctagcctccttcagcctcctcctgggcccaggcaggaagctgaatgaggggggctcactctttaagaggagcagcccacatgaagagcatgtgggtgcctatgcccggtcctcatgatccccgtgagacagaggcagcctcgtgacctggctcccaggctgctcagcgtggtatgcacaaaagccacctccctttgaagtggtccccacctcccctgccccagccaggcctttcagtgctgcaaatgtcagcccactttgcataattgagacaattgggcataatcattctttcagaagcccccactggcaggcagcttatgccccagccctcatgagccaggaagaggagccacgtgcttccaattactgcggagcctttttaagttggtcagagttgggccagaggttgcgacgactccgacggcaaacgctgagtgatgacctgagagtggtaagttgaaataaaccatttctttcccaacctgcttttcatcatggtattttatctgcaccatagaaacattaagacatagcccaacaaggggccttgggcaccagtgctgaaggttctcacatttcaccttgctggatccccaaatcctcatcatgtgcccaccccaaaccctctgcagtcaccactttctcaaagtagattttacttccaattgccatttgctaaatctgcctcctaaaaaccttgcggggggagtagggattaaggctgattacagatgttacagaagctatgtagtctctgagcactgggtgggagtccagccggagggtgagaagcagtccagctccttctgagctgactgagccatcaatatcatctcaaactctgagccctgctgtccagtctcataaagaggactctcttacctcagctgaccagggcctcccatgcagcaggctggacctcacagggaatgcagaagcacccatggggtccatgaggaag

SEQ ID NO: 42 - DNA, 1070 bp, synthetic construct; identical to SEQ ID NO: 41
  source 1..1070: mol_type = other DNA

SEQ ID NO: 43 - DNA, 1248 bp, synthetic construct
  source 1..1248: mol_type = other DNA
atggtgagcaagggcgaggagctgttcaccggggtggtgcccatcctggtcgagctggacggcgacgtaaacggccacaagttcagcgtgtccggcgagggcgagggcgatgccacctacggcaagctgaccctgaagttcatctgcaccaccggcaagctgcccgtgccctggcccaccctcgtgaccaccctgacctacggcgtgcagtgcttcagccgctaccccgaccacatgaagcagcacgacttcttcaagtccgccatgcccgaaggctacgtccaggagcgcaccatcttcttcaaggacgacggcaactacaagacccgcgccgaggtgaagttcgagggcgacaccctggtgaaccgcatcgagctgaagggcatcgacttcaaggaggacggcaacatcctggggcacaagctggagtacaactacaacagccacaacgtctatatcatggccgacaagcagaagaacggcatcaaggtgaacttcaagatccgccacaacatcgaggacggcagcgtgcagctcgccgaccactaccagcagaacacccccatcggcgacggccccgtgctgctgcccgacaaccactacctgagcacccagtccgccctgagcaaagaccccaacgagaagcgcgatcacatggtcctgctggagttcgtgaccgccgccgggatcactctcggcatggacgagctgtacaaggatatctccggaggtatggtcttcacactcgaagatttcgttggggactggcgacagacagccggctacaacctggaccaagtccttgaacagggaggtgtgtccagtttgtttcagaatctcggggtgtccgtaactccgatccaaaggattgtcctgagcggtgaaaatgggctgaagatcgacatccatgtcatcatcccgtatgaaggtctgagcggcgaccaaatgggccagatcgaaaaaatttttaaggtggtgtaccctgtggatgatcatcactttaaggtgatcctgcactatggcacactggtaatcgacggggttacgccgaacatgatcgactatttcggacggccgtatgaaggcatcgccgtgttcgacggcaaaaagatcactgtaacagggaccctgtggaacggcaacaaaattatcgacgagcgcctgatcaaccccgacggctccctgctgttccgagtaaccatcaacggagtgaccggctggcggctgtgcgaacgcattctggcgtaa

SEQ ID NO: 44 - protein, 415 aa, synthetic construct
MVSKGEELFTGVVPILVELDGDVNGHKFSVSGEGEGDATYGKLTLKFICTTGKLPVPWPTLVTTLTYGVQCFSRYPDHMKQHDFFKSAMPEGYVQERTIFFKDDGNYKTRAEVKFEGDTLVNRIELKGIDFKEDGNILGHKLEYNYNSHNVYIMADKQKNGIKVNFKIRHNIEDGSVQLADHYQQNTPIGDGPVLLPDNHYLSTQSALSKDPNEKRDHMVLLEFVTAAGITLGMDELYKDISGGMVFTLEDFVGDWRQTAGYNLDQVLEQGGVSSLFQNLGVSVTPIQRIVLSGENGLKIDIHVIIPYEGLSGDQMGQIEKIFKVVYPVDDHHFKVILHYGTLVIDGVTPNMIDYFGRPYEGIAVFDGKKITVTGTLWNGNKIIDERLINPDGSLLFRVTINGVTGWRLCERILA

SEQ ID NO: 45 - skipped

SEQ ID NO: 46 - DNA, 1137 bp, synthetic construct
  source 1..1137: mol_type = other DNA
atgcgaccccaaatactcctcttgctggctttgttgacccttggactggctaacggaacagaaggtcccaacttctacgttcctttcagcaataagacaggcgtagtcagatccatgggcttccagctcaatccggaatacctgaacgaaacaattttgctggacgactgtacgccaatctatctgaacgtcggtcccctgtgggagcaaaaggttgcccgaggtacgcaatggtttggtgttatcctctcgttggcgtttctcatctattatatatggataacatataaggcgacttgcggatgggaagaactgtacgtgtgtacgatcgaattttgtaaaattgtaattgaactctacttcgagttttcgcctccggcgatgatatatcagaccaacggagaggtaacgccctggttgcgatatgctgaatggctcttgacctgcccagtcatttgcatacatttgagtaacattacaggactcaatgacgactattcgggccgaactatgtccctgatcacatccgacctgggaggcatctgcatggccgttacttccgccttgagtaaaggctggttgaagtggctctttttcgtgatcggctgttgttacggtgctagtacgttttatcatgcggcgctcatatatatagaaagttactacactatgcctcacggtgtttgtaaaaacatggtattggcgatggcagcggtattttttacaagttggttcatgtttcccggtttgttcctggcaggccctgaaggaaccaatgcactgtcgtgggcgggctcgactatcggtcataccgtggcagatttgctctccaaaaacgcctggggtatgattggtcacttcctccgactggagatacacaaacatataattattcatggtgatgttcgtcgcccgataacggttaataccttgggacgagaagtcacggtgtcgtgttttgtcgataaagaagaggaggatgaagacgaacgtatcagcactaagacctacgcgaaccgggcactcgagaaatccagaattacttctgaaggggagtatatccctctggatcaaatagacatcaatgttgtcgacactagttctagatctagattttgctatgaaaatgaagtttaa

SEQ ID NO: 47 - protein, 378 aa, synthetic construct
MRPQILLLLALLTLGLANGTEGPNFYVPFSNKTGVVRSMGFQLNPEYLNETILLDDCTPIYLNVGPLWEQKVARGTQWFGVILSLAFLIYYIWITYKATCGWEELYVCTIEFCKIVIELYFEFSPPAMIYQTNGEVTPWLRYAEWLLTCPVICIHLSNITGLNDDYSGRTMSLITSDLGGICMAVTSALSKGWLKWLFFVIGCCYGASTFYHAALIYIESYYTMPHGVCKNMVLAMAAVFFTSWFMFPGLFLAGPEGTNALSWAGSTIGHTVADLLSKNAWGMIGHFLRLEIHKHIIIHGDVRRPITVNTLGREVTVSCFVDKEEEDEDERISTKTYANRALEKSRITSEGEYIPLDQIDINVVDTSSRSRFCYENEV